European Patent Application EP 4 461 128 A2, published November 13, 2024. Title: NOVEL INSECT RESISTANT GENES AND METHODS OF USE. Applicant: BASF SE. The sequence listing filed with the application follows.

SEQUENCE LISTING (42 sequences)

SEQ ID NO: 1 - DNA, 948 bp, synthetic construct
  misc_feature 1..948: note = Variant: Axmi486-V162A
  source 1..948: mol_type = other DNA
atgctggctgttgctgccaagacagagaacaacaaggagcagcaagtgatcacccacttcaaccagagggagaacaagttccctgatgttggccaaggaatccaatggctctctcagttctatgggaaatcattgaagaacaatggagaaggatattctcttggccaagatgtgatgagatacttcttggaggtgaagaacagctatgggcagcttgcaatggagcctcaggtcatctcaacaactcctctctgggctggccaaagtgatttggagaatgcaacagatcatgagcaaaccctcaactcaacagagttcaagaagacatacagcaacaccacaacaacctccacagagaatggcttcatgattggccaagaaacagaagggaaggttgggattccctttgttgctgaagggaaggtcaccatcaagacagagtacaacttcaatcacaccaatggctatgaaacttcagagagtgctgaatatattgctccaagccaaagcatcaaggttcctcctcacaccattgcaagggtgactgctctgctggatgtgaagaagatcaaggggaagatgcacctctattcagagattggcttgaacaaggattatggctatgacatggtgccactggtgtacaagtatggaggccccttcaagtatgtcacccttggaaccctctatgatgaaggctacaagcaagctcagctggattacttcaacatggggaatgtgattccagaagagattgaaactgtttcaaagagcaacaacccaaaccacttgctggcttctggtgttgggatctttgagagtgaatatggaagtgtcttcaatgtgaaggtggaatacatcaacattaacaccaagaagattgagaagacagagaatctcaccattgagccaaccattgtgccagtgaagcagaccaacaccaagtaa

SEQ ID NO: 2 - DNA, 948 bp, synthetic construct
  misc_feature 1..948: note = Variant: Axmi486-V162A R60A
  source 1..948: mol_type = other DNA
atgctggctgttgctgccaagacagagaacaacaaggagcagcaagtgatcacccacttcaaccagagggagaacaagttccctgatgttggccaaggaatccaatggctctctcagttctatgggaaatcattgaagaacaatggagaaggatattctcttggccaagatgtgatggcgtacttcttggaggtgaagaacagctatgggcagcttgcaatggagcctcaggtcatctcaacaactcctctctgggctggccaaagtgatttggagaatgcaacagatcatgagcaaaccctcaactcaacagagttcaagaagacatacagcaacaccacaacaacctccacagagaatggcttcatgattggccaagaaacagaagggaaggttgggattccctttgttgctgaagggaaggtcaccatcaagacagagtacaacttcaatcacaccaatggctatgaaacttcagagagtgctgaatatattgctccaagccaaagcatcaaggttcctcctcacaccattgcaagggtgactgctctgctggatgtgaagaagatcaaggggaagatgcacctctattcagagattggcttgaacaaggattatggctatgacatggtgccactggtgtacaagtatggaggccccttcaagtatgtcacccttggaaccctctatgatgaaggctacaagcaagctcagctggattacttcaacatggggaatgtgattccagaagagattgaaactgtttcaaagagcaacaacccaaaccacttgctggcttctggtgttgggatctttgagagtgaatatggaagtgtcttcaatgtgaaggtggaatacatcaacattaacaccaagaagattgagaagacagagaatctcaccattgagccaaccattgtgccagtgaagcagaccaacaccaagtaa

SEQ ID NO: 3 - DNA, 948 bp, synthetic construct
  misc_feature 1..948: note = Variant: Axmi486-D96P
  source 1..948: mol_type = other DNA
atgctggctgttgctgccaagacagagaacaacaaggagcagcaagtgatcacccacttcaaccagagggagaacaagttccctgatgttggccaaggaatccaatggctctctcagttctatgggaaatcattgaagaacaatggagaaggatattctcttggccaagatgtgatgagatacttcttggaggtgaagaacagctatgggcagcttgcaatggagcctcaggtcatctcaacaactcctctctgggctggccaaagtgatttggagaatgcaacaccgcatgagcaaaccctcaactcaacagagttcaagaagacatacagcaacaccacaacaacctccacagagaatggcttcatgattggccaagaaacagaagggaaggttgggattccctttgttgctgaagggaaggtcaccatcaagacagagtacaacttcaatcacaccaatggctatgaaacttcagagagtgtggaatatattgctccaagccaaagcatcaaggttcctcctcacaccattgcaagggtgactgctctgctggatgtgaagaagatcaaggggaagatgcacctctattcagagattggcttgaacaaggattatggctatgacatggtgccactggtgtacaagtatggaggccccttcaagtatgtcacccttggaaccctctatgatgaaggctacaagcaagctcagctggattacttcaacatggggaatgtgattccagaagagattgaaactgtttcaaagagcaacaacccaaaccacttgctggcttctggtgttgggatctttgagagtgaatatggaagtgtcttcaatgtgaaggtggaatacatcaacattaacaccaagaagattgagaagacagagaatctcaccattgagccaaccattgtgccagtgaagcagaccaacaccaagtaa

SEQ ID NO: 4 - DNA, 948 bp, synthetic construct
  misc_feature 1..948: note = Variant: Axmi486-H97D
  source 1..948: mol_type = other DNA
atgctggctgttgctgccaagacagagaacaacaaggagcagcaagtgatcacccacttcaaccagagggagaacaagttccctgatgttggccaaggaatccaatggctctctcagttctatgggaaatcattgaagaacaatggagaaggatattctcttggccaagatgtgatgagatacttcttggaggtgaagaacagctatgggcagcttgcaatggagcctcaggtcatctcaacaactcctctctgggctggccaaagtgatttggagaatgcaacagatgatgagcaaaccctcaactcaacagagttcaagaagacatacagcaacaccacaacaacctccacagagaatggcttcatgattggccaagaaacagaagggaaggttgggattccctttgttgctgaagggaaggtcaccatcaagacagagtacaacttcaatcacaccaatggctatgaaacttcagagagtgtggaatatattgctccaagccaaagcatcaaggttcctcctcacaccattgcaagggtgactgctctgctggatgtgaagaagatcaaggggaagatgcacctctattcagagattggcttgaacaaggattatggctatgacatggtgccactggtgtacaagtatggaggccccttcaagtatgtcacccttggaaccctctatgatgaaggctacaagcaagctcagctggattacttcaacatggggaatgtgattccagaagagattgaaactgtttcaaagagcaacaacccaaaccacttgctggcttctggtgttgggatctttgagagtgaatatggaagtgtcttcaatgtgaaggtggaatacatcaacattaacaccaagaagattgagaagacagagaatctcaccattgagccaaccattgtgccagtgaagcagaccaacaccaagtaa

SEQ ID NO: 5 - DNA, 948 bp, synthetic construct
  misc_feature 1..948: note = Variant: Axmi486-H97L
  source 1..948: mol_type = other DNA
atgctggctgttgctgccaagacagagaacaacaaggagcagcaagtgatcacccacttcaaccagagggagaacaagttccctgatgttggccaaggaatccaatggctctctcagttctatgggaaatcattgaagaacaatggagaaggatattctcttggccaagatgtgatgagatacttcttggaggtgaagaacagctatgggcagcttgcaatggagcctcaggtcatctcaacaactcctctctgggctggccaaagtgatttggagaatgcaacagatctggagcaaaccctcaactcaacagagttcaagaagacatacagcaacaccacaacaacctccacagagaatggcttcatgattggccaagaaacagaagggaaggttgggattccctttgttgctgaagggaaggtcaccatcaagacagagtacaacttcaatcacaccaatggctatgaaacttcagagagtgtggaatatattgctccaagccaaagcatcaaggttcctcctcacaccattgcaagggtgactgctctgctggatgtgaagaagatcaaggggaagatgcacctctattcagagattggcttgaacaaggattatggctatgacatggtgccactggtgtacaagtatggaggccccttcaagtatgtcacccttggaaccctctatgatgaaggctacaagcaagctcagctggattacttcaacatggggaatgtgattccagaagagattgaaactgtttcaaagagcaacaacccaaaccacttgctggcttctggtgttgggatctttgagagtgaatatggaagtgtcttcaatgtgaaggtggaatacatcaacattaacaccaagaagattgagaagacagagaatctcaccattgagccaaccattgtgccagtgaagcagaccaacaccaagtaa

SEQ ID NO: 6 - DNA, 948 bp, synthetic construct
  misc_feature 1..948: note = Variant: Axmi486-T100N
  source 1..948: mol_type = other DNA
atgctggctgttgctgccaagacagagaacaacaaggagcagcaagtgatcacccacttcaaccagagggagaacaagttccctgatgttggccaaggaatccaatggctctctcagttctatgggaaatcattgaagaacaatggagaaggatattctcttggccaagatgtgatgagatacttcttggaggtgaagaacagctatgggcagcttgcaatggagcctcaggtcatctcaacaactcctctctgggctggccaaagtgatttggagaatgcaacagatcatgagcaaaatctcaactcaacagagttcaagaagacatacagcaacaccacaacaacctccacagagaatggcttcatgattggccaagaaacagaagggaaggttgggattccctttgttgctgaagggaaggtcaccatcaagacagagtacaacttcaatcacaccaatggctatgaaacttcagagagtgtggaatatattgctccaagccaaagcatcaaggttcctcctcacaccattgcaagggtgactgctctgctggatgtgaagaagatcaaggggaagatgcacctctattcagagattggcttgaacaaggattatggctatgacatggtgccactggtgtacaagtatggaggccccttcaagtatgtcacccttggaaccctctatgatgaaggctacaagcaagctcagctggattacttcaacatggggaatgtgattccagaagagattgaaactgtttcaaagagcaacaacccaaaccacttgctggcttctggtgttgggatctttgagagtgaatatggaagtgtcttcaatgtgaaggtggaatacatcaacattaacaccaagaagattgagaagacagagaatctcaccattgagccaaccattgtgccagtgaagcagaccaacaccaagtaa

SEQ ID NO: 7 - DNA, 948 bp, synthetic construct
  misc_feature 1..948: note = Variant: Axmi486-T100P
  source 1..948: mol_type = other DNA
atgctggctgttgctgccaagacagagaacaacaaggagcagcaagtgatcacccacttcaaccagagggagaacaagttccctgatgttggccaaggaatccaatggctctctcagttctatgggaaatcattgaagaacaatggagaaggatattctcttggccaagatgtgatgagatacttcttggaggtgaagaacagctatgggcagcttgcaatggagcctcaggtcatctcaacaactcctctctgggctggccaaagtgatttggagaatgcaacagatcatgagcaaccgctcaactcaacagagttcaagaagacatacagcaacaccacaacaacctccacagagaatggcttcatgattggccaagaaacagaagggaaggttgggattccctttgttgctgaagggaaggtcaccatcaagacagagtacaacttcaatcacaccaatggctatgaaacttcagagagtgtggaatatattgctccaagccaaagcatcaaggttcctcctcacaccattgcaagggtgactgctctgctggatgtgaagaagatcaaggggaagatgcacctctattcagagattggcttgaacaaggattatggctatgacatggtgccactggtgtacaagtatggaggccccttcaagtatgtcacccttggaaccctctatgatgaaggctacaagcaagctcagctggattacttcaacatggggaatgtgattccagaagagattgaaactgtttcaaagagcaacaacccaaaccacttgctggcttctggtgttgggatctttgagagtgaatatggaagtgtcttcaatgtgaaggtggaatacatcaacattaacaccaagaagattgagaagacagagaatctcaccattgagccaaccattgtgccagtgaagcagaccaacaccaagtaa

SEQ ID NO: 8 - DNA, 948 bp, synthetic construct
  misc_feature 1..948: note = Variant: Axmi486-T100N D96P
  source 1..948: mol_type = other DNA
atgctggctgttgctgccaagacagagaacaacaaggagcagcaagtgatcacccacttcaaccagagggagaacaagttccctgatgttggccaaggaatccaatggctctctcagttctatgggaaatcattgaagaacaatggagaaggatattctcttggccaagatgtgatgagatacttcttggaggtgaagaacagctatgggcagcttgcaatggagcctcaggtcatctcaacaactcctctctgggctggccaaagtgatttggagaatgcaacaccgcatgagcaaaatctcaactcaacagagttcaagaagacatacagcaacaccacaacaacctccacagagaatggcttcatgattggccaagaaacagaagggaaggttgggattccctttgttgctgaagggaaggtcaccatcaagacagagtacaacttcaatcacaccaatggctatgaaacttcagagagtgtggaatatattgctccaagccaaagcatcaaggttcctcctcacaccattgcaagggtgactgctctgctggatgtgaagaagatcaaggggaagatgcacctctattcagagattggcttgaacaaggattatggctatgacatggtgccactggtgtacaagtatggaggccccttcaagtatgtcacccttggaaccctctatgatgaaggctacaagcaagctcagctggattacttcaacatggggaatgtgattccagaagagattgaaactgtttcaaagagcaacaacccaaaccacttgctggcttctggtgttgggatctttgagagtgaatatggaagtgtcttcaatgtgaaggtggaatacatcaacattaacaccaagaagattgagaagacagagaatctcaccattgagccaaccattgtgccagtgaagcagaccaacaccaagtaa

SEQ ID NO: 9 - DNA, 948 bp, synthetic construct
  misc_feature 1..948: note = Variant: Axmi486-D96P H97D
  source 1..948: mol_type = other DNA
atgctggctgttgctgccaagacagagaacaacaaggagcagcaagtgatcacccacttcaaccagagggagaacaagttccctgatgttggccaaggaatccaatggctctctcagttctatgggaaatcattgaagaacaatggagaaggatattctcttggccaagatgtgatgagatacttcttggaggtgaagaacagctatgggcagcttgcaatggagcctcaggtcatctcaacaactcctctctgggctggccaaagtgatttggagaatgcaacaccggatgagcaaaccctcaactcaacagagttcaagaagacatacagcaacaccacaacaacctccacagagaatggcttcatgattggccaagaaacagaagggaaggttgggattccctttgttgctgaagggaaggtcaccatcaagacagagtacaacttcaatcacaccaatggctatgaaacttcagagagtgtggaatatattgctccaagccaaagcatcaaggttcctcctcacaccattgcaagggtgactgctctgctggatgtgaagaagatcaaggggaagatgcacctctattcagagattggcttgaacaaggattatggctatgacatggtgccactggtgtacaagtatggaggccccttcaagtatgtcacccttggaaccctctatgatgaaggctacaagcaagctcagctggattacttcaacatggggaatgtgattccagaagagattgaaactgtttcaaagagcaacaacccaaaccacttgctggcttctggtgttgggatctttgagagtgaatatggaagtgtcttcaatgtgaaggtggaatacatcaacattaacaccaagaagattgagaagacagagaatctcaccattgagccaaccattgtgccagtgaagcagaccaacaccaagtaa

SEQ ID NO: 10 - DNA, 948 bp, synthetic construct
  misc_feature 1..948: note = Variant: Axmi486-D96P H97L
  source 1..948: mol_type = other DNA
atgctggctgttgctgccaagacagagaacaacaaggagcagcaagtgatcacccacttcaaccagagggagaacaagttccctgatgttggccaaggaatccaatggctctctcagttctatgggaaatcattgaagaacaatggagaaggatattctcttggccaagatgtgatgagatacttcttggaggtgaagaacagctatgggcagcttgcaatggagcctcaggtcatctcaacaactcctctctgggctggccaaagtgatttggagaatgcaacaccgctggagcaaaccctcaactcaacagagttcaagaagacatacagcaacaccacaacaacctccacagagaatggcttcatgattggccaagaaacagaagggaaggttgggattccctttgttgctgaagggaaggtcaccatcaagacagagtacaacttcaatcacaccaatggctatgaaacttcagagagtgtggaatatattgctccaagccaaagcatcaaggttcctcctcacaccattgcaagggtgactgctctgctggatgtgaagaagatcaaggggaagatgcacctctattcagagattggcttgaacaaggattatggctatgacatggtgccactggtgtacaagtatggaggccccttcaagtatgtcacccttggaaccctctatgatgaaggctacaagcaagctcagctggattacttcaacatggggaatgtgattccagaagagattgaaactgtttcaaagagcaacaacccaaaccacttgctggcttctggtgttgggatctttgagagtgaatatggaagtgtcttcaatgtgaaggtggaatacatcaacattaacaccaagaagattgagaagacagagaatctcaccattgagccaaccattgtgccagtgaagcagaccaacaccaagtaa

SEQ ID NO: 11 - DNA, 948 bp, synthetic construct
  misc_feature 1..948: note = Variant: Axmi486-H97L T100N D96P
  source 1..948: mol_type = other DNA
atgctggctgttgctgccaagacagagaacaacaaggagcagcaagtgatcacccacttcaaccagagggagaacaagttccctgatgttggccaaggaatccaatggctctctcagttctatgggaaatcattgaagaacaatggagaaggatattctcttggccaagatgtgatgagatacttcttggaggtgaagaacagctatgggcagcttgcaatggagcctcaggtcatctcaacaactcctctctgggctggccaaagtgatttggagaatgcaacaccgctggagcaaaatctcaactcaacagagttcaagaagacatacagcaacaccacaacaacctccacagagaatggcttcatgattggccaagaaacagaagggaaggttgggattccctttgttgctgaagggaaggtcaccatcaagacagagtacaacttcaatcacaccaatggctatgaaacttcagagagtgtggaatatattgctccaagccaaagcatcaaggttcctcctcacaccattgcaagggtgactgctctgctggatgtgaagaagatcaaggggaagatgcacctctattcagagattggcttgaacaaggattatggctatgacatggtgccactggtgtacaagtatggaggccccttcaagtatgtcacccttggaaccctctatgatgaaggctacaagcaagctcagctggattacttcaacatggggaatgtgattccagaagagattgaaactgtttcaaagagcaacaacccaaaccacttgctggcttctggtgttgggatctttgagagtgaatatggaagtgtcttcaatgtgaaggtggaatacatcaacattaacaccaagaagattgagaagacagagaatctcaccattgagccaaccattgtgccagtgaagcagaccaacaccaagtaa

SEQ ID NO: 12 - DNA, 948 bp, synthetic construct
  misc_feature 1..948: note = Variant: Axmi486-T100P D96P
  source 1..948: mol_type = other DNA
atgctggctgttgctgccaagacagagaacaacaaggagcagcaagtgatcacccacttcaaccagagggagaacaagttccctgatgttggccaaggaatccaatggctctctcagttctatgggaaatcattgaagaacaatggagaaggatattctcttggccaagatgtgatgagatacttcttggaggtgaagaacagctatgggcagcttgcaatggagcctcaggtcatctcaacaactcctctctgggctggccaaagtgatttggagaatgcaacaccgcatgagcaaccgctcaactcaacagagttcaagaagacatacagcaacaccacaacaacctccacagagaatggcttcatgattggccaagaaacagaagggaaggttgggattccctttgttgctgaagggaaggtcaccatcaagacagagtacaacttcaatcacaccaatggctatgaaacttcagagagtgtggaatatattgctccaagccaaagcatcaaggttcctcctcacaccattgcaagggtgactgctctgctggatgtgaagaagatcaaggggaagatgcacctctattcagagattggcttgaacaaggattatggctatgacatggtgccactggtgtacaagtatggaggccccttcaagtatgtcacccttggaaccctctatgatgaaggctacaagcaagctcagctggattacttcaacatggggaatgtgattccagaagagattgaaactgtttcaaagagcaacaacccaaaccacttgctggcttctggtgttgggatctttgagagtgaatatggaagtgtcttcaatgtgaaggtggaatacatcaacattaacaccaagaagattgagaagacagagaatctcaccattgagccaaccattgtgccagtgaagcagaccaacaccaagtaa

SEQ ID NO: 13 - DNA, 948 bp, synthetic construct
  misc_feature 1..948: note = Variant: Axmi486-T100P H97D
  source 1..948: mol_type = other DNA
atgctggctgttgctgccaagacagagaacaacaaggagcagcaagtgatcacccacttcaaccagagggagaacaagttccctgatgttggccaaggaatccaatggctctctcagttctatgggaaatcattgaagaacaatggagaaggatattctcttggccaagatgtgatgagatacttcttggaggtgaagaacagctatgggcagcttgcaatggagcctcaggtcatctcaacaactcctctctgggctggccaaagtgatttggagaatgcaacagatgatgagcaaccgctcaactcaacagagttcaagaagacatacagcaacaccacaacaacctccacagagaatggcttcatgattggccaagaaacagaagggaaggttgggattccctttgttgctgaagggaaggtcaccatcaagacagagtacaacttcaatcacaccaatggctatgaaacttcagagagtgtggaatatattgctccaagccaaagcatcaaggttcctcctcacaccattgcaagggtgactgctctgctggatgtgaagaagatcaaggggaagatgcacctctattcagagattggcttgaacaaggattatggctatgacatggtgccactggtgtacaagtatggaggccccttcaagtatgtcacccttggaaccctctatgatgaaggctacaagcaagctcagctggattacttcaacatggggaatgtgattccagaagagattgaaactgtttcaaagagcaacaacccaaaccacttgctggcttctggtgttgggatctttgagagtgaatatggaagtgtcttcaatgtgaaggtggaatacatcaacattaacaccaagaagattgagaagacagagaatctcaccattgagccaaccattgtgccagtgaagcagaccaacaccaagtaa

SEQ ID NO: 14 - DNA, 948 bp, synthetic construct
  misc_feature 1..948: note = Variant: Axmi486-T100N H97D
  source 1..948: mol_type = other DNA
atgctggctgttgctgccaagacagagaacaacaaggagcagcaagtgatcacccacttcaaccagagggagaacaagttccctgatgttggccaaggaatccaatggctctctcagttctatgggaaatcattgaagaacaatggagaaggatattctcttggccaagatgtgatgagatacttcttggaggtgaagaacagctatgggcagcttgcaatggagcctcaggtcatctcaacaactcctctctgggctggccaaagtgatttggagaatgcaacagatgatgagcaaaatctcaactcaacagagttcaagaagacatacagcaacaccacaacaacctccacagagaatggcttcatgattggccaagaaacagaagggaaggttgggattccctttgttgctgaagggaaggtcaccatcaagacagagtacaacttcaatcacaccaatggctatgaaacttcagagagtgtggaatatattgctccaagccaaagcatcaaggttcctcctcacaccattgcaagggtgactgctctgctggatgtgaagaagatcaaggggaagatgcacctctattcagagattggcttgaacaaggattatggctatgacatggtgccactggtgtacaagtatggaggccccttcaagtatgtcacccttggaaccctctatgatgaaggctacaagcaagctcagctggattacttcaacatggggaatgtgattccagaagagattgaaactgtttcaaagagcaacaacccaaaccacttgctggcttctggtgttgggatctttgagagtgaatatggaagtgtcttcaatgtgaaggtggaatacatcaacattaacaccaagaagattgagaagacagagaatctcaccattgagccaaccattgtgccagtgaagcagaccaacaccaagtaa

SEQ ID NO: 15 - DNA, 948 bp, synthetic construct
  misc_feature 1..948: note = Variant: Axmi486-T100N H97L
  source 1..948: mol_type = other DNA
atgctggctgttgctgccaagacagagaacaacaaggagcagcaagtgatcacccacttcaaccagagggagaacaagttccctgatgttggccaaggaatccaatggctctctcagttctatgggaaatcattgaagaacaatggagaaggatattctcttggccaagatgtgatgagatacttcttggaggtgaagaacagctatgggcagcttgcaatggagcctcaggtcatctcaacaactcctctctgggctggccaaagtgatttggagaatgcaacagatctggagcaaaatctcaactcaacagagttcaagaagacatacagcaacaccacaacaacctccacagagaatggcttcatgattggccaagaaacagaagggaaggttgggattccctttgttgctgaagggaaggtcaccatcaagacagagtacaacttcaatcacaccaatggctatgaaacttcagagagtgtggaatatattgctccaagccaaagcatcaaggttcctcctcacaccattgcaagggtgactgctctgctggatgtgaagaagatcaaggggaagatgcacctctattcagagattggcttgaacaaggattatggctatgacatggtgccactggtgtacaagtatggaggccccttcaagtatgtcacccttggaaccctctatgatgaaggctacaagcaagctcagctggattacttcaacatggggaatgtgattccagaagagattgaaactgtttcaaagagcaacaacccaaaccacttgctggcttctggtgttgggatctttgagagtgaatatggaagtgtcttcaatgtgaaggtggaatacatcaacattaacaccaagaagattgagaagacagagaatctcaccattgagccaaccattgtgccagtgaagcagaccaacaccaagtaa

SEQ ID NO: 16 - DNA, 948 bp, synthetic construct
  misc_feature 1..948: note = Variant: Axmi486-H97D T100P D96P
  source 1..948: mol_type = other DNA
atgctggctgttgctgccaagacagagaacaacaaggagcagcaagtgatcacccacttcaaccagagggagaacaagttccctgatgttggccaaggaatccaatggctctctcagttctatgggaaatcattgaagaacaatggagaaggatattctcttggccaagatgtgatgagatacttcttggaggtgaagaacagctatgggcagcttgcaatggagcctcaggtcatctcaacaactcctctctgggctggccaaagtgatttggagaatgcaacaccggatgagcaaccgctcaactcaacagagttcaagaagacatacagcaacaccacaacaacctccacagagaatggcttcatgattggccaagaaacagaagggaaggttgggattccctttgttgctgaagggaaggtcaccatcaagacagagtacaacttcaatcacaccaatggctatgaaacttcagagagtgtggaatatattgctccaagccaaagcatcaaggttcctcctcacaccattgcaagggtgactgctctgctggatgtgaagaagatcaaggggaagatgcacctctattcagagattggcttgaacaaggattatggctatgacatggtgccactggtgtacaagtatggaggccccttcaagtatgtcacccttggaaccctctatgatgaaggctacaagcaagctcagctggattacttcaacatggggaatgtgattccagaagagattgaaactgtttcaaagagcaacaacccaaaccacttgctggcttctggtgttgggatctttgagagtgaatatggaagtgtcttcaatgtgaaggtggaatacatcaacattaacaccaagaagattgagaagacagagaatctcaccattgagccaaccattgtgccagtgaagcagaccaacaccaagtaa

SEQ ID NO: 17 - DNA, 948 bp, synthetic construct
  misc_feature 1..948: note = Variant: Axmi486-H97L T100P D96P
  source 1..948: mol_type = other DNA
atgctggctgttgctgccaagacagagaacaacaaggagcagcaagtgatcacccacttcaaccagagggagaacaagttccctgatgttggccaaggaatccaatggctctctcagttctatgggaaatcattgaagaacaatggagaaggatattctcttggccaagatgtgatgagatacttcttggaggtgaagaacagctatgggcagcttgcaatggagcctcaggtcatctcaacaactcctctctgggctggccaaagtgatttggagaatgcaacaccgctggagcaaccgctcaactcaacagagttcaagaagacatacagcaacaccacaacaacctccacagagaatggcttcatgattggccaagaaacagaagggaaggttgggattccctttgttgctgaagggaaggtcaccatcaagacagagtacaacttcaatcacaccaatggctatgaaacttcagagagtgtggaatatattgctccaagccaaagcatcaaggttcctcctcacaccattgcaagggtgactgctctgctggatgtgaagaagatcaaggggaagatgcacctctattcagagattggcttgaacaaggattatggctatgacatggtgccactggtgtacaagtatggaggccccttcaagtatgtcacccttggaaccctctatgatgaaggctacaagcaagctcagctggattacttcaacatggggaatgtgattccagaagagattgaaactgtttcaaagagcaacaacccaaaccacttgctggcttctggtgttgggatctttgagagtgaatatggaagtgtcttcaatgtgaaggtggaatacatcaacattaacaccaagaagattgagaagacagagaatctcaccattgagccaaccattgtgccagtgaagcagaccaacaccaagtaa

SEQ ID NO: 18 - DNA, 948 bp, synthetic construct
  misc_feature 1..948: note = Variant: Axmi486-H97D T100N D96P
  source 1..948: mol_type = other DNA
atgctggctgttgctgccaagacagagaacaacaaggagcagcaagtgatcacccacttcaaccagagggagaacaagttccctgatgttggccaaggaatccaatggctctctcagttctatgggaaatcattgaagaacaatggagaaggatattctcttggccaagatgtgatgagatacttcttggaggtgaagaacagctatgggcagcttgcaatggagcctcaggtcatctcaacaactcctctctgggctggccaaagtgatttggagaatgcaacaccggatgagcaaaatctcaactcaacagagttcaagaagacatacagcaacaccacaacaacctccacagagaatggcttcatgattggccaagaaacagaagggaaggttgggattccctttgttgctgaagggaaggtcaccatcaagacagagtacaacttcaatcacaccaatggctatgaaacttcagagagtgtggaatatattgctccaagccaaagcatcaaggttcctcctcacaccattgcaagggtgactgctctgctggatgtgaagaagatcaaggggaagatgcacctctattcagagattggcttgaacaaggattatggctatgacatggtgccactggtgtacaagtatggaggccccttcaagtatgtcacccttggaaccctctatgatgaaggctacaagcaagctcagctggattacttcaacatggggaatgtgattccagaagagattgaaactgtttcaaagagcaacaacccaaaccacttgctggcttctggtgttgggatctttgagagtgaatatggaagtgtcttcaatgtgaaggtggaatacatcaacattaacaccaagaagattgagaagacagagaatctcaccattgagccaaccattgtgccagtgaagcagaccaacaccaagtaa

SEQ ID NO: 19 - protein, 315 aa, synthetic construct
  REGION 1..315: note = Variant: Axmi486-V162A
MLAVAAKTENNKEQQVITHFNQRENKFPDVGQGIQWLSQFYGKSLKNNGEGYSLGQDVMRYFLEVKNSYGQLAMEPQVISTTPLWAGQSDLENATDHEQTLNSTEFKKTYSNTTTTSTENGFMIGQETEGKVGIPFVAEGKVTIKTEYNFNHTNGYETSESAEYIAPSQSIKVPPHTIARVTALLDVKKIKGKMHLYSEIGLNKDYGYDMVPLVYKYGGPFKYVTLGTLYDEGYKQAQLDYFNMGNVIPEEIETVSKSNNPNHLLASGVGIFESEYGSVFNVKVEYININTKKIEKTENLTIEPTIVPVKQTNTK

SEQ ID NO: 20 - protein, 315 aa, synthetic construct
  REGION 1..315: note = Variant: Axmi486-V162A R60A
MLAVAAKTENNKEQQVITHFNQRENKFPDVGQGIQWLSQFYGKSLKNNGEGYSLGQDVMAYFLEVKNSYGQLAMEPQVISTTPLWAGQSDLENATDHEQTLNSTEFKKTYSNTTTTSTENGFMIGQETEGKVGIPFVAEGKVTIKTEYNFNHTNGYETSESAEYIAPSQSIKVPPHTIARVTALLDVKKIKGKMHLYSEIGLNKDYGYDMVPLVYKYGGPFKYVTLGTLYDEGYKQAQLDYFNMGNVIPEEIETVSKSNNPNHLLASGVGIFESEYGSVFNVKVEYININTKKIEKTENLTIEPTIVPVKQTNTK

SEQ ID NO: 21 - protein, 315 aa, synthetic construct
  REGION 1..315: note = Variant: Axmi486-D96P
MLAVAAKTENNKEQQVITHFNQRENKFPDVGQGIQWLSQFYGKSLKNNGEGYSLGQDVMRYFLEVKNSYGQLAMEPQVISTTPLWAGQSDLENATPHEQTLNSTEFKKTYSNTTTTSTENGFMIGQETEGKVGIPFVAEGKVTIKTEYNFNHTNGYETSESVEYIAPSQSIKVPPHTIARVTALLDVKKIKGKMHLYSEIGLNKDYGYDMVPLVYKYGGPFKYVTLGTLYDEGYKQAQLDYFNMGNVIPEEIETVSKSNNPNHLLASGVGIFESEYGSVFNVKVEYININTKKIEKTENLTIEPTIVPVKQTNTK

SEQ ID NO: 22 - protein, 315 aa, synthetic construct
  REGION 1..315: note = Variant: Axmi486-H97D
MLAVAAKTENNKEQQVITHFNQRENKFPDVGQGIQWLSQFYGKSLKNNGEGYSLGQDVMRYFLEVKNSYGQLAMEPQVISTTPLWAGQSDLENATDDEQTLNSTEFKKTYSNTTTTSTENGFMIGQETEGKVGIPFVAEGKVTIKTEYNFNHTNGYETSESVEYIAPSQSIKVPPHTIARVTALLDVKKIKGKMHLYSEIGLNKDYGYDMVPLVYKYGGPFKYVTLGTLYDEGYKQAQLDYFNMGNVIPEEIETVSKSNNPNHLLASGVGIFESEYGSVFNVKVEYININTKKIEKTENLTIEPTIVPVKQTNTK

SEQ ID NO: 23 - protein, 315 aa, synthetic construct
  REGION 1..315: note = Variant: Axmi486-H97L
MLAVAAKTENNKEQQVITHFNQRENKFPDVGQGIQWLSQFYGKSLKNNGEGYSLGQDVMRYFLEVKNSYGQLAMEPQVISTTPLWAGQSDLENATDLEQTLNSTEFKKTYSNTTTTSTENGFMIGQETEGKVGIPFVAEGKVTIKTEYNFNHTNGYETSESVEYIAPSQSIKVPPHTIARVTALLDVKKIKGKMHLYSEIGLNKDYGYDMVPLVYKYGGPFKYVTLGTLYDEGYKQAQLDYFNMGNVIPEEIETVSKSNNPNHLLASGVGIFESEYGSVFNVKVEYININTKKIEKTENLTIEPTIVPVKQTNTK

SEQ ID NO: 24 - protein, 315 aa, synthetic construct
  REGION 1..315: note = Variant: Axmi486-T100N
MLAVAAKTENNKEQQVITHFNQRENKFPDVGQGIQWLSQFYGKSLKNNGEGYSLGQDVMRYFLEVKNSYGQLAMEPQVISTTPLWAGQSDLENATDHEQNLNSTEFKKTYSNTTTTSTENGFMIGQETEGKVGIPFVAEGKVTIKTEYNFNHTNGYETSESVEYIAPSQSIKVPPHTIARVTALLDVKKIKGKMHLYSEIGLNKDYGYDMVPLVYKYGGPFKYVTLGTLYDEGYKQAQLDYFNMGNVIPEEIETVSKSNNPNHLLASGVGIFESEYGSVFNVKVEYININTKKIEKTENLTIEPTIVPVKQTNTK

SEQ ID NO: 25 - protein, 315 aa, synthetic construct
  REGION 1..315: note = Variant: Axmi486-T100P
MLAVAAKTENNKEQQVITHFNQRENKFPDVGQGIQWLSQFYGKSLKNNGEGYSLGQDVMRYFLEVKNSYGQLAMEPQVISTTPLWAGQSDLENATDHEQPLNSTEFKKTYSNTTTTSTENGFMIGQETEGKVGIPFVAEGKVTIKTEYNFNHTNGYETSESVEYIAPSQSIKVPPHTIARVTALLDVKKIKGKMHLYSEIGLNKDYGYDMVPLVYKYGGPFKYVTLGTLYDEGYKQAQLDYFNMGNVIPEEIETVSKSNNPNHLLASGVGIFESEYGSVFNVKVEYININTKKIEKTENLTIEPTIVPVKQTNTK

SEQ ID NO: 26 - protein, 315 aa, synthetic construct
  REGION 1..315: note = Variant: Axmi486-T100N D96P
MLAVAAKTENNKEQQVITHFNQRENKFPDVGQGIQWLSQFYGKSLKNNGEGYSLGQDVMRYFLEVKNSYGQLAMEPQVISTTPLWAGQSDLENATPHEQNLNSTEFKKTYSNTTTTSTENGFMIGQETEGKVGIPFVAEGKVTIKTEYNFNHTNGYETSESVEYIAPSQSIKVPPHTIARVTALLDVKKIKGKMHLYSEIGLNKDYGYDMVPLVYKYGGPFKYVTLGTLYDEGYKQAQLDYFNMGNVIPEEIETVSKSNNPNHLLASGVGIFESEYGSVFNVKVEYININTKKIEKTENLTIEPTIVPVKQTNTK

SEQ ID NO: 27 - protein, 315 aa, synthetic construct
  REGION 1..315: note = Variant: Axmi486-D96P H97D
MLAVAAKTENNKEQQVITHFNQRENKFPDVGQGIQWLSQFYGKSLKNNGEGYSLGQDVMRYFLEVKNSYGQLAMEPQVISTTPLWAGQSDLENATPDEQTLNSTEFKKTYSNTTTTSTENGFMIGQETEGKVGIPFVAEGKVTIKTEYNFNHTNGYETSESVEYIAPSQSIKVPPHTIARVTALLDVKKIKGKMHLYSEIGLNKDYGYDMVPLVYKYGGPFKYVTLGTLYDEGYKQAQLDYFNMGNVIPEEIETVSKSNNPNHLLASGVGIFESEYGSVFNVKVEYININTKKIEKTENLTIEPTIVPVKQTNTK

SEQ ID NO: 28 - protein, 315 aa, synthetic construct
  REGION 1..315: note = Variant: Axmi486-D96P H97L
MLAVAAKTENNKEQQVITHFNQRENKFPDVGQGIQWLSQFYGKSLKNNGEGYSLGQDVMRYFLEVKNSYGQLAMEPQVISTTPLWAGQSDLENATPLEQTLNSTEFKKTYSNTTTTSTENGFMIGQETEGKVGIPFVAEGKVTIKTEYNFNHTNGYETSESVEYIAPSQSIKVPPHTIARVTALLDVKKIKGKMHLYSEIGLNKDYGYDMVPLVYKYGGPFKYVTLGTLYDEGYKQAQLDYFNMGNVIPEEIETVSKSNNPNHLLASGVGIFESEYGSVFNVKVEYININTKKIEKTENLTIEPTIVPVKQTNTK

SEQ ID NO: 29 - protein, 315 aa, synthetic construct
  REGION 1..315: note = Variant: Axmi486-H97L T100N D96P
MLAVAAKTENNKEQQVITHFNQRENKFPDVGQGIQWLSQFYGKSLKNNGEGYSLGQDVMRYFLEVKNSYGQLAMEPQVISTTPLWAGQSDLENATPLEQNLNSTEFKKTYSNTTTTSTENGFMIGQETEGKVGIPFVAEGKVTIKTEYNFNHTNGYETSESVEYIAPSQSIKVPPHTIARVTALLDVKKIKGKMHLYSEIGLNKDYGYDMVPLVYKYGGPFKYVTLGTLYDEGYKQAQLDYFNMGNVIPEEIETVSKSNNPNHLLASGVGIFESEYGSVFNVKVEYININTKKIEKTENLTIEPTIVPVKQTNTK

SEQ ID NO: 30 - protein, 315 aa, synthetic construct
  REGION 1..315: note = Variant: Axmi486-T100P D96P
MLAVAAKTENNKEQQVITHFNQRENKFPDVGQGIQWLSQFYGKSLKNNGEGYSLGQDVMRYFLEVKNSYGQLAMEPQVISTTPLWAGQSDLENATPHEQPLNSTEFKKTYSNTTTTSTENGFMIGQETEGKVGIPFVAEGKVTIKTEYNFNHTNGYETSESVEYIAPSQSIKVPPHTIARVTALLDVKKIKGKMHLYSEIGLNKDYGYDMVPLVYKYGGPFKYVTLGTLYDEGYKQAQLDYFNMGNVIPEEIETVSKSNNPNHLLASGVGIFESEYGSVFNVKVEYININTKKIEKTENLTIEPTIVPVKQTNTK

SEQ ID NO: 31 - protein, 315 aa, synthetic construct
  REGION 1..315: note = Variant: Axmi486-T100P H97D
MLAVAAKTENNKEQQVITHFNQRENKFPDVGQGIQWLSQFYGKSLKNNGEGYSLGQDVMRYFLEVKNSYGQLAMEPQVISTTPLWAGQSDLENATDDEQPLNSTEFKKTYSNTTTTSTENGFMIGQETEGKVGIPFVAEGKVTIKTEYNFNHTNGYETSESVEYIAPSQSIKVPPHTIARVTALLDVKKIKGKMHLYSEIGLNKDYGYDMVPLVYKYGGPFKYVTLGTLYDEGYKQAQLDYFNMGNVIPEEIETVSKSNNPNHLLASGVGIFESEYGSVFNVKVEYININTKKIEKTENLTIEPTIVPVKQTNTK

SEQ ID NO: 32 - protein, 315 aa, synthetic construct
  REGION 1..315: note = Variant: Axmi486-T100N H97D
MLAVAAKTENNKEQQVITHFNQRENKFPDVGQGIQWLSQFYGKSLKNNGEGYSLGQDVMRYFLEVKNSYGQLAMEPQVISTTPLWAGQSDLENATDDEQNLNSTEFKKTYSNTTTTSTENGFMIGQETEGKVGIPFVAEGKVTIKTEYNFNHTNGYETSESVEYIAPSQSIKVPPHTIARVTALLDVKKIKGKMHLYSEIGLNKDYGYDMVPLVYKYGGPFKYVTLGTLYDEGYKQAQLDYFNMGNVIPEEIETVSKSNNPNHLLASGVGIFESEYGSVFNVKVEYININTKKIEKTENLTIEPTIVPVKQTNTK

SEQ ID NO: 33 - protein, 315 aa, synthetic construct
  REGION 1..315: note = Variant: Axmi486-T100N H97L
MLAVAAKTENNKEQQVITHFNQRENKFPDVGQGIQWLSQFYGKSLKNNGEGYSLGQDVMRYFLEVKNSYGQLAMEPQVISTTPLWAGQSDLENATDLEQNLNSTEFKKTYSNTTTTSTENGFMIGQETEGKVGIPFVAEGKVTIKTEYNFNHTNGYETSESVEYIAPSQSIKVPPHTIARVTALLDVKKIKGKMHLYSEIGLNKDYGYDMVPLVYKYGGPFKYVTLGTLYDEGYKQAQLDYFNMGNVIPEEIETVSKSNNPNHLLASGVGIFESEYGSVFNVKVEYININTKKIEKTENLTIEPTIVPVKQTNTK

SEQ ID NO: 34 - protein, 315 aa, synthetic construct
  REGION 1..315: note = Variant: Axmi486-H97D T100P D96P
MLAVAAKTENNKEQQVITHFNQRENKFPDVGQGIQWLSQFYGKSLKNNGEGYSLGQDVMRYFLEVKNSYGQLAMEPQVISTTPLWAGQSDLENATPDEQPLNSTEFKKTYSNTTTTSTENGFMIGQETEGKVGIPFVAEGKVTIKTEYNFNHTNGYETSESVEYIAPSQSIKVPPHTIARVTALLDVKKIKGKMHLYSEIGLNKDYGYDMVPLVYKYGGPFKYVTLGTLYDEGYKQAQLDYFNMGNVIPEEIETVSKSNNPNHLLASGVGIFESEYGSVFNVKVEYININTKKIEKTENLTIEPTIVPVKQTNTK

SEQ ID NO: 35 - protein, 315 aa, synthetic construct
  REGION 1..315: note = Variant: Axmi486-H97L T100P D96P
MLAVAAKTENNKEQQVITHFNQRENKFPDVGQGIQWLSQFYGKSLKNNGEGYSLGQDVMRYFLEVKNSYGQLAMEPQVISTTPLWAGQSDLENATPLEQPLNSTEFKKTYSNTTTTSTENGFMIGQETEGKVGIPFVAEGKVTIKTEYNFNHTNGYETSESVEYIAPSQSIKVPPHTIARVTALLDVKKIKGKMHLYSEIGLNKDYGYDMVPLVYKYGGPFKYVTLGTLYDEGYKQAQLDYFNMGNVIPEEIETVSKSNNPNHLLASGVGIFESEYGSVFNVKVEYININTKKIEKTENLTIEPTIVPVKQTNTK

SEQ ID NO: 36 - protein, 315 aa, synthetic construct
  REGION 1..315: note = Variant: Axmi486-H97D T100N D96P
MLAVAAKTENNKEQQVITHFNQRENKFPDVGQGIQWLSQFYGKSLKNNGEGYSLGQDVMRYFLEVKNSYGQLAMEPQVISTTPLWAGQSDLENATPDEQNLNSTEFKKTYSNTTTTSTENGFMIGQETEGKVGIPFVAEGKVTIKTEYNFNHTNGYETSESVEYIAPSQSIKVPPHTIARVTALLDVKKIKGKMHLYSEIGLNKDYGYDMVPLVYKYGGPFKYVTLGTLYDEGYKQAQLDYFNMGNVIPEEIETVSKSNNPNHLLASGVGIFESEYGSVFNVKVEYININTKKIEKTENLTIEPTIVPVKQTNTK

SEQ ID NO: 37 - DNA, 1023 bp, Bacillus thuringiensis
  misc_feature 1..1023: note = axmi-486 (Ref: WO/2015/088937)
  source 1..1023: mol_type = unassigned DNA
gtgagggagaaggatttgaataaaaaagtaacaaaggcagtattaagcatgatagtgggtataagtgttttagcatctcctttagctgtagccgcaaaaacagagaataataaagaacaacaagtaattacacattttaatcagagagaaaataagttccctgatgtaggacaggggattcaatggttatctcaattttatggaaagtctttaaagaataatggtgaaggatactccttaggtcaggatgtaatgagatattttttagaagtaaagaattcttacggtcaattggcaatggaacctcaagtaataagcactacacctctttgggccggccaaagtgacttggaaaatgcaactgatcatgaacaaactttaaattccacagaatttaaaaaaacgtattctaacacaacaaccacctctacagaaaatggatttatgataggtcaagagactgaagggaaagttggtattccctttgtcgcagaaggaaaagtcaccataaaaactgaatataactttaatcatactaatgggtatgaaacatctgaaagtgtagagtatattgctccttctcaatctattaaggtaccaccgcatactattgcccgagtgacagcattattagatgtgaaaaaaatcaaagggaaaatgcatctatattcagaaattgggcttaataaagattatggttacgatatggtgccacttgtttataaatatggaggtccatttaagtatgtaaccttaggcacattatatgacgagggctataagcaggcacaattagattatttcaatatgggaaatgttataccggaagaaattgagactgtttcaaaaagtaacaatcccaaccatttattagcaagtggagtaggaatctttgaatcagaatacggaagtgtatttaatgttaaagttgaatacattaatattaatacgaaaaagattgaaaaaacagagaatcttactattgaacctacaatagtccctgttaaacagacgaatacaaaa

SEQ ID NO: 38 - protein, 341 aa, Bacillus thuringiensis
  REGION 1..341: note = axmi-486 (Ref: WO/2015/088937)
MREKDLNKKVTKAVLSMIVGISVLASPLAVAAKTENNKEQQVITHFNQRENKFPDVGQGIQWLSQFYGKSLKNNGEGYSLGQDVMRYFLEVKNSYGQLAMEPQVISTTPLWAGQSDLENATDHEQTLNSTEFKKTYSNTTTTSTENGFMIGQETEGKVGIPFVAEGKVTIKTEYNFNHTNGYETSESVEYIAPSQSIKVPPHTIARVTALLDVKKIKGKMHLYSEIGLNKDYGYDMVPLVYKYGGPFKYVTLGTLYDEGYKQAQLDYFNMGNVIPEEIETVSKSNNPNHLLASGVGIFESEYGSVFNVKVEYININTKKIEKTENLTIEPTIVPVKQTNTK

SEQ ID NO: 39 - protein, 325 aa, Bacillus thuringiensis
  REGION 1..325: note = axmi-486 (alternate start site) (Ref: WO/2015/088937)
MIVGISVLASPLAVAAKTENNKEQQVITHFNQRENKFPDVGQGIQWLSQFYGKSLKNNGEGYSLGQDVMRYFLEVKNSYGQLAMEPQVISTTPLWAGQSDLENATDHEQTLNSTEFKKTYSNTTTTSTENGFMIGQETEGKVGIPFVAEGKVTIKTEYNFNHTNGYETSESVEYIAPSQSIKVPPHTIARVTALLDVKKIKGKMHLYSEIGLNKDYGYDMVPLVYKYGGPFKYVTLGTLYDEGYKQAQLDYFNMGNVIPEEIETVSKSNNPNHLLASGVGIFESEYGSVFNVKVEYININTKKIEKTENLTIEPTIVPVKQTNTK

SEQ ID NO: 40 - protein, 315 aa, Bacillus thuringiensis
  REGION 1..315: note = axmi-486 (alternate start site) (Ref: WO/2015/088937)
MLAVAAKTENNKEQQVITHFNQRENKFPDVGQGIQWLSQFYGKSLKNNGEGYSLGQDVMRYFLEVKNSYGQLAMEPQVISTTPLWAGQSDLENATDHEQTLNSTEFKKTYSNTTTTSTENGFMIGQETEGKVGIPFVAEGKVTIKTEYNFNHTNGYETSESVEYIAPSQSIKVPPHTIARVTALLDVKKIKGKMHLYSEIGLNKDYGYDMVPLVYKYGGPFKYVTLGTLYDEGYKQAQLDYFNMGNVIPEEIETVSKSNNPNHLLASGVGIFESEYGSVFNVKVEYININTKKIEKTENLTIEPTIVPVKQTNTK

SEQ ID NO: 41 - protein, 257 aa, Bacillus thuringiensis
  REGION 1..257: note = axmi-486 (alternate start site) (Ref: WO/2015/088937)
MRYFLEVKNSYGQLAMEPQVISTTPLWAGQSDLENATDHEQTLNSTEFKKTYSNTTTTSTENGFMIGQETEGKVGIPFVAEGKVTIKTEYNFNHTNGYETSESVEYIAPSQSIKVPPHTIARVTALLDVKKIKGKMHLYSEIGLNKDYGYDMVPLVYKYGGPFKYVTLGTLYDEGYKQAQLDYFNMGNVIPEEIETVSKSNNPNHLLASGVGIFESEYGSVFNVKVEYININTKKIEKTENLTIEPTIVPVKQTNTK

SEQ ID NO: 42 - protein, 242 aa, Bacillus thuringiensis
  REGION 1..242: note = axmi-486 (alternate start site) (Ref: WO/2015/088937)
MEPQVISTTPLWAGQSDLENATDHEQTLNSTEFKKTYSNTTTTSTENGFMIGQETEGKVGIPFVAEGKVTIKTEYNFNHTNGYETSESVEYIAPSQSIKVPPHTIARVTALLDVKKIKGKMHLYSEIGLNKDYGYDMVPLVYKYGGPFKYVTLGTLYDEGYKQAQLDYFNMGNVIPEEIETVSKSNNPNHLLASGVGIFESEYGSVFNVKVEYININTKKIEKTENLTIEPTIVPVKQTNTK